European Patent Application EP 4 293 104 A2, published December 20, 2023. Title: CELL-FREE PRODUCTION OF RIBONUCLEIC ACID. Applicant: GreenLight Biosciences, Inc. Application EP. The sequence listing filed with the application follows.

SEQUENCE LISTING (28 sequences)

SEQ ID NO: 1 - protein, 813 aa, Escherichia coli
MSQDPFQEREAEKYANPIPSREFILEHLTKREKPASRDELAVELHIEGEEQLEGLRRRLRAMERDGQLVFTRRQCYALPERLDLVKGTVIGHRDGYGFLRVEGRKDDLYLSSEQMKTCIHGDQVLAQPLGADRKGRREARIVRVLVPKTSQIVGRYFTEAGVGFVVPDDSRLSFDILIPPDQIMGARMGFVVVVELTQRPTRRTKAVGKIVEVLGDNMGTGMAVDIALRTHEIPYIWPQAVEQQVAGLKEEVPEEAKAGRVDLRDLPLVTIDGEDARDFDDAVYCEKKRGGGWRLWVAIADVSYYVRPSTPLDREARNRGTSVYFPSQVIPMLPEVLSNGLCSLNPQVDRLCMVCEMTVSSKGRLTGYKFYEAVMSSHARLTYTKVWHILQGDQDLREQYAPLVKHLEELHNLYKVLDKAREERGGISFESEEAKFIFNAERRIERIEQTQRNDAHKLIEECMILANISAARFVEKAKEPALFRIHDKPSTEAITSFRSVLAELGLELPGGNKPEPRDYAELLESVADRPDAEMLQTMLLRSMKQAIYDPENRGHFGLALQSYAHFTSPIRRYPDLTLHRAIKYLLAKEQGHQGNTTETGGYHYSMEEMLQLGQHCSMAERRADEATRDVADWLKCDFMLDQVGNVFKGVISSVTGFGFFVRLDDLFIDGLVHVSSLDNDYYRFDQVGQRLMGESSGQTYRLGDRVEVRVEAVNMDERKIDFSLISSERAPRNVGKTAREKAKKGDAGKKGGKRRQVGKKVNFEPDSAFRGEKKTKPKAAKKDARKAKKPSAKTQKIAAATKAKRAAKKKVAE

SEQ ID NO: 2 - protein, 732 aa, Thermosynechococcus elongatus
MPSAKSPRRKAPEPIDLDNPQYYFNRSLSWLEFNKRVLHEAYDPRTPLLERLKFMAIFSSNLDEFFMVRVAGLKQQVESGILQVGADGMPPAEQLQAVRQYLLPIVTEQHRYFDQELRALLAKESIFLTRFNELTPEQQAYLNDYFQAQVFPVLTPLAVDPAHPFPYISSLSLNLAVLIRDPESGQERLARVKVPNQFPRFVALPQHLHSPQGVHWLGVPLEEIIAHNLSALFPGMEIEAYFAFRITRSADLELETDKADDLLIAIEQEIRKRRFGSVVRLEVQRGIPPLLRQTLMEEMDLEEIDVYELEGLLCLNDLFAFMGLPLPQFKDPEWQPQVPPSFQRVEERESMFDTSSEITTLGTDYWEAVANELFSLIREGDIIVHHPYHSFAATVQRFITLAAHDPQVLAIKITLYRTSGDSPIVSALIKAAENGKQVAVLVELKARFDEENNILWARKLEKVGVHVVYGVPGLKTHTKTVLVVRQEAGQIRRYVHIGTGNYNPKTASLYEDLGLFSCREELGADLSELFNVLTGYARQRDYRKLLVAPVTMRDRTLQLIYREIEHARNGQPARIIAKMNAITDTQVIRALYEASQAGVDIDLIIRGMCCLRPGVPGVSDRIRVISIIGRFLEHSRIFYFGNNGDPEYYIGSADWRSRNLDRRVEAITPIEDPAIQLELKERLEIMLADNRQAWELQPDGTYRQRQPAPGEAERGTHSVLMARTLKDVQGSH

SEQ ID NO: 3 - protein, 225 aa, Pyrococcus furiosus
MRIVFDIGGSVLVPENPDIDFIKEIAYQLTKVSEDHEVAVVVGGGKLARKYIEVAEKFNSSETFKDFIGIQITRANAMLLIAALREKAYPVVVEDFWEAWKAVQLKKIPVMGGTHPGHTTDAVAALLAEFLKADLLVVITNVDGVYTADPKKDPTAKKIKKMKPEELLEIVGKGIEKAGSSSVIDPLAAKIIARSGIKTIVIGKEDAKDLFRVIKGDHNGTTIEP

SEQ ID NO: 4 - protein, 208 aa, Thermus thermophilus
MRGIVTIDGPSASGKSSVARRVAAALGVPYLSSGLLYRAAAFLALRAGVDPGDEEGLLALLEGLGVRLLAQAEGNRVLADGEDLTSFLHTPEVDRVVSAVARLPGVRAWVNRRLKEVPPPFVAEGRDMGTAVFPEAAHKFYLTASPEVRAWRRARERPQAYEEVLRDLLRRDERDKAQSAPAPDALVLDTGGMTLDEVVAWVLAHIRR

SEQ ID NO: 5 - protein, 207 aa, Thermatoga maritima [sequence omitted]

SEQ ID NO: 6 - protein, 186 aa, Thermus thermophilus
MDVGQAVIFLGPPGAGKGTQASRLAQELGFKKLSTGDILRDHVARGTPLGERVRPIMERGDLVPDDLILELIREELAERVIFDGFPRTLAQAEALDRLLSETGTRLLGVVLVEVPEEELVRRILRRAELEGRSDDNEETVRRRLEVYREKTEPLVGYYEARGVLKRVDGLGTPDEVYARIRAALGI

SEQ ID NO: 7 - protein, 142 aa, Aquifex aeolicus
MAVERTLIIVKPDAMEKGALGKILDRFIQEGFQIKALKMFRFTPEKAGEFYYVHRERPFFQELVEFMSSGPVVAAVLEGEDAIKRVREIIGPTDSEEARKVAPNSIRAQFGTDKGKNAIHASDSPESAQYEICFIFSGLEIV

SEQ ID NO: 8 - protein, 280 aa, Meiothermus ruber
MGFCSIEFLMGAQMKKYRVQPDGRFELKRFDPDDTSAFEGGKQAALEALAVLNRRLEKLQELLYAEGQHKVLVVLQAMDAGGKDGTIRVVFDGVNPSGVRVASFGVPTEQELARDYLWRVHQQVPRKGELVIFNRSHYEDVLVVRVKNLVPQQVWQKRYRHIREFERMLADEGTTILKFFLHISKDEQRQRLQERLDNPEKRWKFRMGDLEDRRLWDRYQEAYEAAIRETSTEYAPWYVIPANKNWYRNWLVSHILVETLEGLAMQYPQPETASEKIVIE

SEQ ID NO: 9 - protein, 268 aa, Meiothermus silvanus
MAKTIGATLNLQDIDPRSTPGFNGDKEKALALLEKLTARLDELQEQLYAEHQHRVLVILQGMDTSGKDGTIRHVFKNVDPLGVRVVAFKAPTPPELERDYLWRVHQHVPANGELVIFNRSHYEDVLVARVHNLVPPAIWSRRYDHINAFEKMLVDEGTTVLKFFLHISKEEQKKRLLERLVEADKHWKFDPQDLVERGYWEDYMEAYQDVLDKTHTQYAPWHVIPADRKWYRNLQVSRLLVEALEGLRMKYPRPKLNIPRLKSELEKM

SEQ ID NO: 10 - protein, 266 aa, Deinococcus geothermalis
MQLDRYRVPPGQRVRLSNWPTDDDGGLSKAEGEALLPDLQQRLANLQERLYAESQQALLIVLQARDAGGKDGTVKHVIGAFNPSGVQVSNFKVPTEEERAHDFLWRIHRQTPRLGMIGVFNRSQYEDVLVTRVHHLIDDQTAQRRLKHICAFESLLTDSGTRIVKFYLHISPEEQKKRLEARLADPSKHWKFNPGDLQERAHWDAYTAVYEDVLTTSTPAAPWYVVPADRKWFRNLLVSQILVQTLEEMNPQFPAPAFNAADLRIV

SEQ ID NO: 11 - protein, 300 aa, Thermosynechococcus elongatus
MIPQDFLDEINPDRYIVPAGGNFHWKDYDPGDTAGLKSKVEAQELLAAGIKKLAAYQDVLYAQNIYGLLIIFQAMDAAGKDSTIKHVMSGLNPQACRVYSFKAPSAEELDHDFLWRANRALPERGCIGIFNRSYYEEVLVVRVHPDLLNRQQLPPETKTKHIWKERFEDINHYERYLTRNGILILKFFLHISKAEQKKRFLERISRPEKNWKFSIEDVRDRAHWDDYQQAYADVFRHTSTKWAPWHIIPANHKWFARLMVAHFIYQKLASLNLHYPMLSEAHREQLLEAKALLENEPDED

SEQ ID NO: 12 - protein, 281 aa, Anaerolinea thermophila
MGEAMERYFIKPGEKVRLKDWSPDPPKDFEGDKESTRAAVAELNRKLEVLQERLYAERKHKVLVILQGMDTSGKDGVIRSVFEGVNPQGVKVANFKVPTQEELDHDYLWRVHKVVPGKGEIVIFNRSHYEDVLVVRVHNLVPPEVWKKRYEQINQFERLLHETGTTILKFFLFISREEQKQRLLERLADPAKHWKFNPGDLKERALWEEYEKAYEDVLSRTSTEYAPWILVPADKKWYRDWVISRVLVETLEGLEIQLPPPLADAETYRRQLLEEDAPESR

SEQ ID NO: 13 - protein, 270 aa, Caldilinea aerophila
MDVDRYRVPPGSTIHLSQWPPDDRSLYEGDKKQGKQDLSALNRRLETLQELLYAEGKHKVLIILQGMDTSGKDGVIRHVFNGVNPQGVKVASFKVPTAVELAHDFLWRIHRQTPGSGEIVIFNRSHYEDVLVVRVHGLVPPEVWARRYEHINAFEKLLVDEGTTILKFFLHISKEEQRQRLLERLEMPEKRWKFSVGDLAERKRWDEYMAAYEAVLSKTSTEYAPWYIVPSDRKWYRNLVISHVIINALEGLNMRYPQPEDIAFDTIVIE

SEQ ID NO: 14 - protein, 294 aa, Chlorobaculum tepidum
MKLDLDAFRIQPGKKPNLAKRPTRIDPVYRSKGEYHELLANHVAELSKLQNVLYADNRYAILLIFQAMDAAGKDSAIKHVMSGVNPQGCQVYSFKHPSATELEHDFLWRTNCVLPERGRIGIFNRSYYEEVLVVRVHPEILEMQNIPHNLAHNGKVWDHRYRSIVSHEQHLHCNGTRIVKFYLHLSKEEQRKRFLERIDDPNKNWKFSTADLEERKFWDQYMEAYESCLQETSTKDSPWFAVPADDKKNARLIVSRIVLDTLESLNLKYPEPSPERRKELLDIRKRLENPENGK

SEQ ID NO: 15 - protein, 269 aa, Oceanithermus profundus
MDVSRYRVPPGSGFDPEAWPTREDDDFAGGKKEAKKELARLAVRLGELQARLYAEGRQALLIVLQGMDTAGKDGTIRHVFRAVNPQGVRVTSFKKPTALELAHDYLWRVHRHAPARGEIGIFNRSHYEDVLVVRVHELVPPEVWGRRYDHINAFERLLADEGTRIVKFFLHISKDEQKRRLEARLENPRKHWKFNPADLSERARWGDYAAAYAEALSRTSSDRAPWYAVPADRKWQRNRIVAQVLVDALEAMDPRFPRVDFDPASVRVE

SEQ ID NO: 16 - protein, 290 aa, Roseiflexus castenholzii
MYAQRVVPGMRVRLHDIDPDANGGLNKDEGRARFAELNAELDVMQEELYAAGIHALLLILQGMDTAGKDGAIRNVMLNLNPQGCRVESFKVPTEEELAHDFLWRVHRVVPRKGMVGVFNRSHYEDVLVVRVHSLVPESVWRARYDQINAFERLLADTGTIIVKCFLHISKEEQEQRLLARERDVSKAWKLSAGDWRERAFWDDYMAAYEEALTRCSTDYAPWYIIPANRKWYRDLAISEALVETLRPYRDDWRRALDAMSRARRAELEAFRAEQHAMEGRPQGAGGVSRR

SEQ ID NO: 17 - protein, 282 aa, Roseiflexus sp.
MHYAHTVIPGTQVRLRDIDPDASGGLTKDEGRERFASFNATLDAMQEELYAAGVHALLLILQGMDTAGKDGAIRNVMHNLNPQGCRVESFKVPTEEELAHDFLWRVHKVVPRKGMVGVFNRSHYEDVLVVRVHSLVPEHVWRARYDQINAFERLLTDTGTIIVKCFLHISKDEQEKRLLAREQDVTKAWKLSAGDWRERERWDEYMAAYEEALTRCSTEYAPWYIIPANRKWYRDLAISEVLVETLRPYRDDWQRALDAMSQARLAELKAFRHQQTAGATRL

SEQ ID NO: 18 - protein, 274 aa, Truepera radiovictrix
MSQGSAKGLGKLDKKVYARELALLQLELVKLQGWIKAQGLKVVVLFEGRDAAGKGSTITRITQPLNPRVCRVVALGAPTERERTQWYFQRYVHHLPAAGEMVLFDRSWYNRAGVERVMGFCTEAEYREFLHACPTFERLLLDAGIILIKYWFSVSAAEQERRMRRRNENPAKRWKLSPMDLEARARWVAYSKAKDAMFYHTDTKASPWYVVNAEDKRRAHLSCIAHLLSLIPYEDLTPPPLEMPPRDLAGADEGYERPDKAHQTWVPDYVPPTR

SEQ ID NO: 19 - protein, 26 aa, synthetic construct
  REGION 1..26: note = Synthetic Polypeptide
MKIKTGARILALSALTTMMFSASALA

SEQ ID NO: 20 - protein, 21 aa, synthetic construct
  REGION 1..21: note = Synthetic Polypeptide
MKQSTIALALLPLLFTPVTKA

SEQ ID NO: 21 - protein, 25 aa, synthetic construct
  REGION 1..25: note = Synthetic Polypeptide
MMITLRKLPLAVAVAAGVMSAQAMA

SEQ ID NO: 22 - protein, 23 aa, synthetic construct
  REGION 1..23: note = Synthetic Polypeptide
MNKKVLTLSAVMASMLFGAAAHA

SEQ ID NO: 23 - protein, 22 aa, synthetic construct
  REGION 1..22: note = Synthetic Polypeptide
MKYLLPTAAAGLLLLAAQPAMA

SEQ ID NO: 24 - protein, 19 aa, synthetic construct
  REGION 1..19: note = Synthetic Polypeptide
MKKIWLALAGLVLAFSASA

SEQ ID NO: 25 - protein, 23 aa, synthetic construct
  REGION 1..23: note = Synthetic Polypeptide
MMTKIKLLMLIIFYLIISASAHA

SEQ ID NO: 26 - protein, 21 aa, synthetic construct
  REGION 1..21: note = Synthetic Polypeptide
MKQALRVAFGFLILWASVLHA

SEQ ID NO: 27 - protein, 18 aa, synthetic construct
  REGION 1..18: note = Synthetic Polypeptide
MRVLLFLLLSLFMLPAFS

SEQ ID NO: 28 - protein, 39 aa, synthetic construct
  REGION 1..39: note = Synthetic Polypeptide
MANNDLFQASRRRFLAQLGGLTVAGMLGPSLLTPRRATA